European Patent Application EP 4 530 294 A1, published April 2, 2025. Title: PREPARATION METHOD FOR BIOSYNTHESIS OF HUMAN BODY STRUCTURAL MATERIAL. Applicant: SHANXI JINBO BIO-PHARMACEUTICAL CO., LTD. Application EP. The sequence listing filed with the application follows.

SEQUENCE LISTING (35 sequences)

SEQ ID NO: 1 - protein, 36 aa, Homo sapiens
GFPGVPGGTGPKGDRGETGSKGEQGLPGERGLRGEP

SEQ ID NO: 2 - protein, 81 aa, Homo sapiens
GLTGPTGAVGLPGPPGPSGLVGPQGSPGLPGQVGETGKPGAPGRDGASGKDGDRGSPGVPGSPGLPGPVGPKGEPGPTGAP

SEQ ID NO: 3 - protein, 48 aa, Homo sapiens
GEPGAKGDRGLPGPRGEKGEAGRAGEPGDPGEDGQKGAPGPKGFKGDP

SEQ ID NO: 4 - protein, 288 aa, synthetic construct
GFPGVPGGTGPKGDRGETGSKGEQGLPGERGLRGEPGFPGVPGGTGPKGDRGETGSKGEQGLPGERGLRGEPGFPGVPGGTGPKGDRGETGSKGEQGLPGERGLRGEPGFPGVPGGTGPKGDRGETGSKGEQGLPGERGLRGEPGFPGVPGGTGPKGDRGETGSKGEQGLPGERGLRGEPGFPGVPGGTGPKGDRGETGSKGEQGLPGERGLRGEPGFPGVPGGTGPKGDRGETGSKGEQGLPGERGLRGEPGFPGVPGGTGPKGDRGETGSKGEQGLPGERGLRGEP

SEQ ID NO: 5 - protein, 324 aa, synthetic construct
GLTGPTGAVGLPGPPGPSGLVGPQGSPGLPGQVGETGKPGAPGRDGASGKDGDRGSPGVPGSPGLPGPVGPKGEPGPTGAPGLTGPTGAVGLPGPPGPSGLVGPQGSPGLPGQVGETGKPGAPGRDGASGKDGDRGSPGVPGSPGLPGPVGPKGEPGPTGAPGLTGPTGAVGLPGPPGPSGLVGPQGSPGLPGQVGETGKPGAPGRDGASGKDGDRGSPGVPGSPGLPGPVGPKGEPGPTGAPGLTGPTGAVGLPGPPGPSGLVGPQGSPGLPGQVGETGKPGAPGRDGASGKDGDRGSPGVPGSPGLPGPVGPKGEPGPTGAP

SEQ ID NO: 6 - protein, 288 aa, synthetic construct
GEPGAKGDRGLPGPRGEKGEAGRAGEPGDPGEDGQKGAPGPKGFKGDPGEPGAKGDRGLPGPRGEKGEAGRAGEPGDPGEDGQKGAPGPKGFKGDPGEPGAKGDRGLPGPRGEKGEAGRAGEPGDPGEDGQKGAPGPKGFKGDPGEPGAKGDRGLPGPRGEKGEAGRAGEPGDPGEDGQKGAPGPKGFKGDPGEPGAKGDRGLPGPRGEKGEAGRAGEPGDPGEDGQKGAPGPKGFKGDPGEPGAKGDRGLPGPRGEKGEAGRAGEPGDPGEDGQKGAPGPKGFKGDP

SEQ ID NO: 7 - DNA, 864 bp, synthetic construct
  source 1..864: mol_type = other DNA
ggatttcccggggtcccgggaggcaccggccctaaaggcgatcgtggtgaaaccggcagcaagggcgagcagggtctgccgggcgagcgcggtttgagaggcgaaccgggttttccaggcgtgccgggcggtacgggtccgaagggtgaccgtggcgaaaccggcagcaagggtgaacaaggtttaccgggtgaacgcggtctgcgtggtgagccgggcttcccaggtgttccgggcggaaccggtcctaaaggtgatcgtggcgaaaccggttccaaaggcgaacaaggtcttccgggtgagcgcggtctgcgtggcgaaccgggtttcccgggcgtgccgggaggcaccggcccaaagggcgaccgcggagaaaccggcagcaaaggcgagcagggcctgccgggtgaacgtggcctgcgtggtgagccgggattcccgggtgttccgggcggcaccggtccgaaaggtgatcgtggtgaaaccggtagcaagggtgaacagggtctgccgggcgagcgcggcttgagaggtgagcctggttttccgggggtgcccggcggtacgggcccgaaaggcgaccgtggcgaaaccggttctaagggtgagcagggtctgccgggtgagcgtggtctgcgcggtgagccgggtttcccgggcgttccgggtggcactggtccgaagggcgaccgtggcgagactggctcgaaaggtgaacagggtttgccgggtgagcgtggtctgcgtggtgagccgggttttccgggcgtgccgggtggcacgggcccaaaaggcgatcgtggtgagaccggttccaagggcgagcaaggtctgccgggcgagcgcggtctccgcggtgaaccg

SEQ ID NO: 8 - DNA, 972 bp, synthetic construct
  source 1..972: mol_type = other DNA
ggactaacagggccgaccggtgcggtcggcctgccgggaccaccgggccccagcggtctggttggtcctcagggttccccgggtcttccgggccaggttggtgagacaggcaagccgggtgcgccgggccgtgacggtgcctctggtaaagacggcgatcgtggttcgccgggcgttccgggttcgccgggtctgccgggtccggtcggtccgaaaggtgaaccggggcccactggtgcgccaggcttgaccggtccgaccggtgcggttggcctcccgggcccaccgggaccgagcggtctggttggcccacaaggttccccgggcttaccgggccaggttggagaaaccggtaagccgggtgcaccggggcgcgacggcgcaagcggtaaggacggcgaccgcggtagcccgggcgtgccgggtagcccgggcctgccgggcccggtgggccccaagggtgagccgggaccgaccggcgctccggggttgaccggtccaacgggcgctgtgggcctgccgggtccaccgggtccgagcggtctggttggcccgcagggtagcccgggtctgccgggccaagttggtgaaaccggtaaaccgggagcaccaggccgtgatggtgcctccggtaaggacggcgatcgcggttctccgggcgtcccgggctccccgggtctgccgggcccggtgggtccgaaaggtgagccgggcccgacgggcgcgccgggcttgaccggcccgacgggtgctgtgggtctgccgggccctccgggtccaagcggtctggtgggccctcaaggttctccgggtctgccgggacaggtgggcgaaaccggtaagccgggtgcgccaggtcgtgatggcgcgagcggcaaagatggtgatcgtggcagtccgggggtgccgggcagcccgggcttgccgggtccagtaggtccgaaaggcgagccgggcccgaccggcgcgcct

SEQ ID NO: 9 - DNA, 864 bp, synthetic construct
  source 1..864: mol_type = other DNA
ggagaacccggggcgaagggcgaccgcggtctgccgggtccgcgtggtgaaaaaggtgaggcgggccgcgcaggcgaaccgggtgacccgggcgaggatggtcagaaaggcgcgccaggtccgaaaggttttaaaggcgatccgggcgaaccgggtgccaagggcgatagaggtctgccgggtccgcgtggcgaaaagggtgaagcgggtcgtgcgggtgaaccgggtgacccgggcgaggacggtcagaagggcgcgccaggtccgaaaggcttcaaaggtgacccgggtgaaccgggcgcgaaaggcgaccgtggtttaccgggtccgcgtggtgagaagggggaggctggtcgtgccggtgaaccgggcgacccaggcgaggatggtcagaaaggcgcgcctggtcccaagggcttcaagggcgacccgggtgaaccgggtgccaaaggggatcgcggtttgccaggtcctcgcggtgaaaagggcgaggctggtcgcgctggtgagccgggcgacccgggtgaagatggtcaaaaaggcgctccgggtccgaagggttttaaaggtgatccgggcgagccgggtgcgaagggcgatcgtggcctgccgggcccacgtggtgagaaaggcgaggccggtcgtgcaggcgaaccgggtgaccccggcgaagatggccaaaagggtgcgcctggcccgaagggattcaaaggcgatccgggtgagccgggcgcgaaaggcgaccgcggcctgccgggtccgcgtggtgagaagggcgaggcaggccgtgcaggtgaaccgggtgacccgggtgaggatggtcaaaaaggtgctccgggtccgaagggctttaagggcgacccg

SEQ ID NO: 10 - protein, 12 aa, synthetic construct
GFPGVPGGTGPK

SEQ ID NO: 11 - protein, 15 aa, synthetic construct
GFPGVPGGTGPKGDR

SEQ ID NO: 12 - protein, 21 aa, synthetic construct
GFPGVPGGTGPKGDRGETGSK

SEQ ID NO: 13 - protein, 18 aa, synthetic construct
GLRGEPGFPGVPGGTGPK

SEQ ID NO: 14 - protein, 21 aa, synthetic construct
GLRGEPGFPGVPGGTGPKGDR

SEQ ID NO: 15 - protein, 15 aa, synthetic construct
GEPGFPGVPGGTGPK

SEQ ID NO: 16 - protein, 18 aa, synthetic construct
GEPGFPGVPGGTGPKGDR

SEQ ID NO: 17 - protein, 24 aa, synthetic construct
GEPGFPGVPGGTGPKGDRGETGSK

SEQ ID NO: 18 - protein, 18 aa, synthetic construct
GDRGETGSKGEQGLPGER

SEQ ID NO: 19 - protein, 15 aa, synthetic construct
GETGSKGEQGLPGER

SEQ ID NO: 20 - protein, 9 aa, synthetic construct
GEQGLPGER

SEQ ID NO: 21 - protein, 288 aa, synthetic construct; identical to SEQ ID NO: 4

SEQ ID NO: 22 - protein, 44 aa, synthetic construct
GLTGPTGAVGLPGPPGPSGLVGPQGSPGLPGQVGETGKPGAPGR

SEQ ID NO: 23 - protein, 28 aa, synthetic construct
DGASGKDGDRGSPGVPGSPGLPGPVGPK

SEQ ID NO: 24 - protein, 22 aa, synthetic construct
DGDRGSPGVPCSPGLPGPVGPK

SEQ ID NO: 25 - protein, 31 aa, synthetic construct
DGDRGSPGVPCSPGLPGPVGPKGEPGPTGAP

SEQ ID NO: 26 - protein, 18 aa, synthetic construct
GSPGVPGSPGLPGPVGPK

SEQ ID NO: 27 - protein, 27 aa, synthetic construct
GSPGVPGSPGLPGPVGPKGEPGPTGAP

SEQ ID NO: 28 - protein, 324 aa, synthetic construct; identical to SEQ ID NO: 5

SEQ ID NO: 29 - protein, 12 aa, synthetic construct
GFKGDPGEPGAK

SEQ ID NO: 30 - protein, 15 aa, synthetic construct
GFKGDPGEPGAKGDR

SEQ ID NO: 31 - protein, 12 aa, synthetic construct
GDPGEPGAKGDR

SEQ ID NO: 32 - protein, 9 aa, synthetic construct
GDRGLPGPR

SEQ ID NO: 33 - protein, 13 aa, synthetic construct
AGEPGDPGEDGQK

SEQ ID NO: 34 - protein, 19 aa, synthetic construct
AGEPGDPGEDGQKGAPGPK

SEQ ID NO: 35 - protein, 273 aa, synthetic construct
GEPGAKGDRGLPGPRGEKGEAGRAGEPGDPGEDGQKGAPGPKGFKGDPGEPGAKGDRGLPGPRGEKGEAGRAGEPGDPGEDGQKGAPGPKGFKGDPGEPGAKGDRGLPGPRGEKGEAGRAGEPGDPGEDGQKGAPGPKGFKGDPGEPGAKGDRGLPGPRGEKGEAGRAGEPGDPGEDGQKGAPGPKGFKGDPGEPGAKGDRGLPGPRGEKGEAGRAGEPGDPGEDGQKGAPGPKGFKGDPGEKGEAGRAGEPGDPGEDGQKGAPGPKGFKGDP